European Patent Application EP 4 471 064 A1, published December 4, 2024. Title: 一种抗原结合蛋白及其用途. Applicant: 明慧医药（杭州）有限公司;. The sequence listing filed with the application follows.

SEQUENCE LISTING (227 sequences)

SEQ ID NO: 1 - protein, 123 aa, synthetic construct
  REGION 1..123: note = 5115
EVQLVESGGGLVQAGGSLRLSCAVSGRTFSSFVMGWFRQAPGKEREFVAAISGSGSRANYADSVKGRFTVSRDNANNTVYLQMNSLKPDDTALYYCAANPRRATPDYTQYAYWGQGTQVTVSS

SEQ ID NO: 2 - protein, 123 aa, synthetic construct
  REGION 1..123: note = 5666
EVQLVESGGGLVQAGGSLRLSCAVSGRTFSSYVMGWFRQAPGKERELVAAISGSGSRSNYADSVKGRFTVSRDNANNTVYLQMSSLRPDDTGLYYCAANPRRATTDYTQYAYWGQGTQVTVSS

SEQ ID NO: 3 - protein, 123 aa, synthetic construct
  REGION 1..123: note = 5115-H0
EVQLVESGGGLVQPGGSLRLSCAASGRTFSSFVMSWFRQAPGKEREFVSAISGSGSRAYYADSVKGRFTISRDNSKNTLYLQMNSLRAEDTAVYYCAANPRRATPDYTQYAYWGQGTQVTVSS

SEQ ID NO: 4 - protein, 123 aa, synthetic construct
  REGION 1..123: note = 5115-H1
EVQLVESGGGLVQPGGSLRLSCAASGRTFSSFVMSWFRQAPGKEREFVSAISGSGSRAYYADSVKGRFTISRDNSKNTLYLQMNSLRAEDTAVYYCAANPRRATPDYTQYAYWGQGTLVTVSS

SEQ ID NO: 5 - protein, 123 aa, synthetic construct
  REGION 1..123: note = 5115-H2
EVQLVESGGGLVQPGGSLRLSCAASGRTFSSFVMSWFRQAPGKGREFVSAISGSGSRAYYADSVKGRFTISRDNSKNTLYLQMNSLRAEDTAVYYCAANPRRATPDYTQYAYWGQGTLVTVSS

SEQ ID NO: 6 - protein, 123 aa, synthetic construct
  REGION 1..123: note = 5115-H3
EVQLVESGGGLVQPGGSLRLSCAASGRTFSSFVMSWFRQAPGKELEFVSAISGSGSRAYYADSVKGRFTISRDNSKNTLYLQMNSLRAEDTAVYYCAANPRRATPDYTQYAYWGQGTLVTVSS

SEQ ID NO: 7 - protein, 123 aa, synthetic construct
  REGION 1..123: note = 5115-H4
EVQLVESGGGLVQPGGSLRLSCAASGRTFSSFVMSWFRQAPGKGLEFVSAISGSGSRAYYADSVKGRFTISRDNSKNTLYLQMNSLRAEDTAVYYCAANPRRATPDYTQYAYWGQGTLVTVSS

SEQ ID NO: 8 - protein, 123 aa, synthetic construct
  REGION 1..123: note = 5115-H5
EVQLVESGGGLVQPGGSLRLSCAASGRTFSSFVMMWFRQAPGKGLEFVSAISGSGSRAYYADSVKGRFTISRDNSKNTLYLQMNSLRAEDTAVYYCAANPRRATPDYTQYAYWGQGTLVTVSS

SEQ ID NO: 9 - protein, 123 aa, synthetic construct
  REGION 1..123: note = 5115-H6
EVQLVESGGGLVQPGGSLRLSCAASGRTFSSFVMMWFRQAPGKEREFVSAISGSGSRAYYADSVKGRFTISRDNSKNTLYLQMNSLRAEDTAVYYCAANPRRATPDYTQYAYWGQGTLVTVSS

SEQ ID NO: 10 - protein, 123 aa, synthetic construct
  REGION 1..123: note = 5115-H4-M3
EVQLVESGGGLVQPGGSLRLSCAASGRTFSSFVMAWFRQAPGKGLEFVSAISGSGSRARYADSVKGRFTISRDNSKNTLYLQMNSLRAEDTAVYYCAANPRRATPDYTQYAYWGQGTLVTVSS

SEQ ID NO: 11 - protein, 123 aa, synthetic construct
  REGION 1..123: note = 5115-H4-M10
EVQLVESGGGLVQPGGSLRLSCAASGRSFSSFVMSWFRQAPGKGLEFVSAISGQGSRSYYADSVKGRFTISRDNSKNTLYLQMNSLRAEDTAVYYCAANPRRATPDLTQYAYWGQGTLVTVSS

SEQ ID NO: 12 - protein, 123 aa, synthetic construct
  REGION 1..123: note = 5115-H4-M12
EVQLVESGGGLVQPGGSLRLSCAASGRTFSSFVMSWFRQAPGKGLEFVSAISGSGSRFYYADSVKGRFTISRDNSKNTLYLQMNSLRAEDTAVYYCAANPRRATPDLTQYAYWGQGTLVTVSS

SEQ ID NO: 13 - protein, 123 aa, synthetic construct
  REGION 1..123: note = 5115-H4-M24
EVQLVESSGGLVQPGGSLRLSCAASGRTFSRFVMSWFRQAPGKGLEFVSAISGSGSRARYADSVKGRFTISRDNSKNTLYLQMNSLRAEDTAVYYCAANPRRATPDLTQYAYWGQGTLVTVSS

SEQ ID NO: 14 - protein, 123 aa, synthetic construct
  REGION 1..123: note = 5115-H4-M25
EVQLVESGGGLVQPGGSLRLSCAASGVTFSSFVMSWFRQAPGKGLEFVSAISGSGSRALYADSVKGRFTISRDNSKNTLYLQMNSLRAEDTAVYYCAANPRRATPDLTQYAYWGQGTLVTVSS

SEQ ID NO: 15 - protein, 123 aa, synthetic construct
  REGION 1..123: note = 5115-H4-M28
EVQLVESGGGLVQPGGSLRLSCAASGRTFSSFVMSWFRQAPGKGLEFVSAISGGGSRAYYADSVKGRFAISRDNSKNTLYLQMNSLRAEDTAVYYCAANPRRATPDLRQYAYWGQGTLVTVSS

SEQ ID NO: 16 - protein, 123 aa, synthetic construct
  REGION 1..123: note = 5115-H4-M34
EVQLVESGGGLVQPGGSLRLSCAASGRTFSSFVMAWFRQAPGKGLEFVSAISGSGSRARYADSVKGRFTISRDNSKNTLYLQMNSLRAEDTAVYYCAANPRRATPDLTQYAYWGQGTLVTVSS

SEQ ID NO: 17 - protein, 123 aa, synthetic construct
  REGION 1..123: note = 5115-H4-M39
EVQLVESGGGLVQPGGSLRLSCAASGRTFSSFVMSWFRQAPGKGLEFVSAISGSGSRSRYADSVKGRFTISRDNSKNTLYLQMNSLRAEDTAVYYCAANPRRATPDLRQYAYWGQGTLVTVSS

SEQ ID NO: 18 - protein, 123 aa, synthetic construct
  REGION 1..123: note = 5115-H4-M41
EVQLVESGGGLVQPGGSLRLSCAASGRTFSSFVMGWFRQAPGKGLEFVSAISGSGSRARYADSVKGRFTISRDNSKNTLYLQMNSLRAEDTAVYYCAANPRRATPDYTQYLYWGQGTLVTVSS

SEQ ID NO: 19 - protein, 123 aa, synthetic construct
  REGION 1..123: note = 5115-H4-M44
EVQLVESGGGLVQPGGSLRLSCAASGRRFSSFVMSWFRQAPGKGLEFVSAISGSGSRARYADSVKGRFTISRDNSKNTLYLQMNSLRAEDTAVYYCAANPRRATPDLTQYAYWGQGTLVTVSS

SEQ ID NO: 20 - protein, 123 aa, synthetic construct
  REGION 1..123: note = 5115-H4-M48
EVQLVESGGGLVQPGDSLRLSCAASGRTFSRFVMSWFRQAPGKGLEFVSAISGSGSRAYYADSVKGRFTISRDNSKNTLYLQMNSLRAEDTAVYYCAANPRRATPDLRQYAYWGQGTLVTVSS

SEQ ID NO: 21 - protein, 123 aa, synthetic construct
  REGION 1..123: note = 5115-H4-M52
EVQLVESGGGLVQPGGSLRLSCAASSRTFSSFVMSWFRQAPGKGLEFVSAISGSGSRANYADSVKGRFTISRDNSKNTLYLQMNSLRAEDTAVYYCAANPRRATPDLTQYAYWGQGTLVTVSS

SEQ ID NO: 22 - protein, 123 aa, synthetic construct
  REGION 1..123: note = 5115-H4-M59
EVQLVESGGGLVQPGGSLRLSCAASGRAFSSFVMSWFRQAPGKGLEFVSAISGRGSRAYYADSVKGRFTISRDNSKNTLYLQMNSLRAEDTAVYYCAANPRRATPDMTQYAYWGQGTLVTVSS

SEQ ID NO: 23 - protein, 123 aa, synthetic construct
  REGION 1..123: note = 5115-H4-M61
EVQLVESGGGLVQPGGSLRLSCAASGRTFSSFVLSWFRQAPGKGLEFVSAISGSGSRARYADSVKGRFTISRDNSKNTLYLQMNSLRAEDTAVYYCAANPRRATPDLTQYAYWGQGTLVTVSS

SEQ ID NO: 24 - protein, 123 aa, synthetic construct
  REGION 1..123: note = 5115-H4-M69
EVQLVESGGGLVQPGGSLRLSCAASGRTFRSFVMSWFRQAPGKGLEFVSAISGSGSRARYADSVKGRFTISRDNSKNTLYLQMNSLRAEDTAVYYCAANPRRATPDLTQYAYWGQGTLVTVSS

SEQ ID NO: 25 - protein, 123 aa, synthetic construct
  REGION 1..123: note = 5115-H1-M1
EVQLVESGGGLVQPGGSLRLSCAASGRTFSSFVMSWFRQAPGKEREFVSAISGSGSRSRYADSVKGRFTISRDNSKNTLYLQMNSLRAEDTAVYYCAANPRRATPDYTQYAYWGQGTLVTVSS

SEQ ID NO: 26 - protein, 123 aa, synthetic construct
  REGION 1..123: note = 5115-H1-M2
EVQLVESGGGLVQPGGSLRLSCAASGRTFSSFVMSWFRQAPGKEREFVSAISGSGSRARYADSVKGRFTISRDNSKNTLYLQMNSLRAEDTAVYYCAANPRRATPDLLQYAYWGQGTLVTVSS

SEQ ID NO: 27 - protein, 123 aa, synthetic construct
  REGION 1..123: note = 5115-H1-M3
EVQLVESGGGLVQPGGSLRLSCAASGRTFSSFVMSWFRQAPGKEREFVSAISGSGSRARYADSVKGRFTISRDNSKNTLYLQMNSLRAEDTAVYYCAANPRRATPDLTQYAYWGQGTLVTVSS

SEQ ID NO: 28 - protein, 123 aa, synthetic construct
  REGION 1..123: note = 5115-H1-M4
EVQLVESGGGLVQPGGSLRLSCAASGRFFSSFVMSWFRQAPGKEREFVSAISGSGSRFRYADSVKGRFTISRDNSKNTLYLQMNSLRAEDTAVYYCAANPRRATPDYTQYAYWGQGTLVTVSS

SEQ ID NO: 29 - protein, 123 aa, synthetic construct
  REGION 1..123: note = 5115-H1-M5
EVQLVESGGGLVQPGGSLRLSCAASGRYFSSFVMAWFRQAPGKGLEFVSAISGSGLRARYADSVKGRFTISRDNSKNTLYLQMNSLRAEDTAVYYCAANPRRATPDLTSYAYWGQGTLVTVSS

SEQ ID NO: 30 - protein, 123 aa, synthetic construct
  REGION 1..123: note = 5115-H1-M6
EVQLVESGGGLVQPGGSLRLSCAASGREFSSFVMAWFRQAPGKGLEFVSAISGSGSRARYADSVKGRFTISRDNSKNTLYLQMNSLRAEDTAVYYCAANPRRATPDLTSYAYWGQGTLVTVSS

SEQ ID NO: 31 - protein, 123 aa, synthetic construct
  REGION 1..123: note = 5115-H1-M7
EVQLVESGGGLVQPGGSLRLSCAASGRTFSSFVMSWFRQAPGKEREFVSAISGRGSRAYYADSVKGRFTISRDNSKNTLYLQMNSLRAEDTAVYYCAANPRRATPDLRQYAYWGQGTLVTVSS

SEQ ID NO: 32 - protein, 123 aa, synthetic construct
  REGION 1..123: note = 5115-H1-M8
EVQLVESGGGLVQPGGSLRLSCAASGRTFSSFVMSWFRQAPGKEREFVSAISGSGSRQRYADSVKGRFTISRDNSKNTLYLQMNSLRAEDTAVYYCAANPRRATPDLSQYAYWGQGTLVTVSS

SEQ ID NO: 33 - protein, 123 aa, synthetic construct
  REGION 1..123: note = 5115-H1-M9
EVQLVESGGGLVQPGGSLRLSCAASGRTFSSFVMSWFRQAPGKEREFVSAISGSGSRLRYADSVKGRFTISRDNSKNTLYLQMNSLRAEDTAVYYCAANPRRATPDLLQYAYWGQGTLVTVSS

SEQ ID NO: 34 - protein, 123 aa, synthetic construct
  REGION 1..123: note = 5115-H1-M10
EVQLVESGGGLVQPGGSLRLSCAASGGTFSSFVMSWFRQAPGKEREFVSAISGSGSRAYYADSVKGRFTISRDNSKNTLYLQMNSLRAEDTAVYYCAANPRRATPGFTQYAYWGQGTLVTVSS

SEQ ID NO: 35 - protein, 123 aa, synthetic construct
  REGION 1..123: note = 5115-H1-M11
EVQLVESGGGLVQPGGSLRLSCAASGIRFSSFVMSWFRQAPGKEREFVSAISGSGSRHRYADSVKGRFTISRDNSKNTLYLQMNSLRAEDTAVYYCAANPRRATPDYTQYAYWGQGTLVTVSS

SEQ ID NO: 36 - protein, 123 aa, synthetic construct
  REGION 1..123: note = 5115-H1-M12
EVQLVESGGGLVQPGGSLRLSCAASGRTFSSFVMSWFRQAPGKEREFVSAISGSGSRARYADSVKGRFTISRDNSKNTLYLQMNSLRAEDTAVYYCAANPRRATPDLRQYAYWGQGTLVTVSS

SEQ ID NO: 37 - protein, 123 aa, synthetic construct
  REGION 1..123: note = 5115-H1-M13
EVQLVESGGGLVQPGGSLRLSCAASLGTFSSFVMSWFRQAPGKEREFVSAISGSGSRARYADSVKGRFTISRDNSKNTLYLQMNSLRAEDTAVYYCAANPRRATPDYTQYAYWGQGTLVTVSS

SEQ ID NO: 38 - protein, 123 aa, synthetic construct
  REGION 1..123: note = 5115-H1-M14
EVQLVESGGGLVQPGGSLRLSCAASGRTFSSFVMSWFRQAPGKEREFVSAISGSGSRMRYADSVKGRFTISRDNSKNTLYLQMNSLRAEDTAVYYCAANPRRATPDLTQYAYWGQGTLVTVSS

SEQ ID NO: 39 - protein, 123 aa, synthetic construct
  REGION 1..123: note = 5115-H1-M15
EVQLVESGGGLVQPGGSLRLSCAASGRTFSSFVMSWFRQAPGKEREFVSAISGSGSRMRYADSVKGRFTISRDNSKNTLYLQMNSLRAEDTAVYYCAANPRRATPDLRQYAYWGQGTLVTVSS

SEQ ID NO: 40 - protein, 123 aa, synthetic construct
  REGION 1..123: note = 5115-H1-M16
EVQLVESGGGLVQPGGSLRLSCAASHRTFSSFVMSWFRQAPGKEREFVSAISGSGSRARYADSVKGRFTISRDNSKNTLYLQMNSLRAEDTAVYYCAANPRRATPDLTQYAYWGQGTLVTVSS

SEQ ID NO: 41 - protein, 123 aa, synthetic construct
  REGION 1..123: note = 5115-H1-M17
EVQLVESGGGLVQPGGSLRLSCAASGRTFSSFVMSWFRQAPGKEREFVSAISGSGSRSRYADSVKGRFTISRDNSKNTLYLQMNSLRAEDTAVYYCAANPRRATPDLIQYAYWGQGTLVTVSS

SEQ ID NO: 42 - protein, 123 aa, synthetic construct
  REGION 1..123: note = 5115-H1-M18
EVQLVESGGGLVQPGGSLRLSCAASGRRFSSFVMSWFRQAPGKEREFVSAISGSGSRARYADSVKGRFTISRDNSKNTLYLQMNSLRAEDTAVYYCAANPRRATPDLTQYAYWGQGTLVTVSS

SEQ ID NO: 43 - protein, 123 aa, synthetic construct
  REGION 1..123: note = 5115-H1-M19
EVQLVESGGGLVQPGGSLRLSCAASGRTFSSFVMSWFRQAPGKEREFVSAISGSGSRMRYADSVKGRFTISRDNSKNTLYLQMNSLRAEDTAVYYCAANPRRATPDLHQYAYWGQGTLVTVSS

SEQ ID NO: 44 - protein, 123 aa, synthetic construct
  REGION 1..123: note = 5115-H1-M20
EVQLVESGGGLVQPGGSLRLSCAASGRTFRSFVMSWFRQAPGKEREFVSAISGSGSRYRYADSVKGRFTISRDNSKNTLYLQMNSLRAEDTAVYYCAANPRRATPDYTQYAYWGQGTLVTVSS

SEQ ID NO: 45 - protein, 123 aa, synthetic construct
  REGION 1..123: note = 5115-H1-M21
EVQLVESGGGLVQPGGSLRLSCAASGKTFSSFVMSWFRQAPGKEREFVSAISGSGSRTRYADSVKGRFTISRDNSKNTLYLQMNSLRAEDTAVYYCAANPRRATPDYTQYAYWGQGTLVTVSS

SEQ ID NO: 46 - protein, 123 aa, synthetic construct
  REGION 1..123: note = 5115-H1-M22
EVQLVESGGGLVQPGGSLRLSCAASGRTFSSFVMSWFRQAPGKEREFVSAISGSGSRSRYADSVKGRFTISRDNSKNTLYLQMNSLRAEDTAVYYCAANPRRATPDLLQYAYWGQGTLVTVSS

SEQ ID NO: 47 - protein, 123 aa, synthetic construct
  REGION 1..123: note = 5115-H1-M23
EVQLVESGGGLVQPGGSLRLSCAASGRTFKSFVMSWFRQAPGKEREFVSAISGSGSRARYADSVKGRFTISRDNSKNTLYLQMNSLRAEDTAVYYCAANPRRATPDMTQYAYWGQGTLVTVSS

SEQ ID NO: 48 - protein, 123 aa, synthetic construct
  REGION 1..123: note = 5115-H1-M24
EVQLVESGGGLVQPGGSLRLSCAASGRTFSGFVMAWFRQAPGKGLEFVSAISGTGSRARYADSVKGRFTISRDNSKNTLYLQMNSLRAEDTAVYYCAANPRRATPDLTQYAYWGQGTLVTVSS

SEQ ID NO: 49 - protein, 123 aa, synthetic construct
  REGION 1..123: note = 5115-H1-M25
EVQLVESGGGLVQPGGSLRLSCAASGRFFSSFVMSWFRQAPGKEREFVSAISGSGSRARYADSVKGRFTISRDNSKNTLYLQMNSLRAEDTAVYYCAANPRRATPDYSQYAYWGQGTLVTVSS

SEQ ID NO: 50 - protein, 123 aa, synthetic construct
  REGION 1..123: note = 5115-H1-M26
EVQLVESGGGLVQPGGSLRLSCAASGRTFSSFVMSWFRQAPGKEREFVSAISGSGSRYTYADSVKGRFTISRDNSKNTLYLQMNSLRAEDTAVYYCAANPRRATPDLMQYAYWGQGTLVTVSS

SEQ ID NO: 51 - protein, 123 aa, synthetic construct
  REGION 1..123: note = 5115-H1-M27
EVQLVESGGGLVQPGGSLRLSCAASGRTLSSFVMAWFRQAPGKGLEFVSAISGSGLRARYADSVKGRFTISRDNSKNTLYLQMNSLRAEDTAVYYCAANPRYATPDLTQYAYWGQGTLVTVSS

SEQ ID NO: 52 - protein, 123 aa, synthetic construct
  REGION 1..123: note = 5115-H1-M28
EVQLVESGGGLVQPGGSLRLSCAASGRTFSSFVMSWFRQAPGKEREFVSAISGSGSRYRYADSVKGRFTISRDNSKNTLYLQMNSLRAEDTAVYYCAANPRRATPDLKQYAYWGQGTLVTVSS

SEQ ID NO: 53 - protein, 123 aa, synthetic construct
  REGION 1..123: note = 5115-H1-M29
EVQLVESGGGLVQPGGSLRLSCAASGRTFSSFVMSWFRQAPGKEREFVSAISGSGSRAYYADSVKGRFTISRDNSKNTLYLQMNSLRAEDTAVYYCAANPRRATPDLRQYAYWGQGTLVTVSS

SEQ ID NO: 54 - protein, 123 aa, synthetic construct
  REGION 1..123: note = 5115-H1-M30
EVQLVESGGGLVQPGGSLRLSCAASGARFSSFVMSWFRQAPGKEREFVSAISGSGSRHRYADSVKGRFTISRDNSKNTLYLQMNSLRAEDTAVYYCAANPRRATPDYTQYAYWGQGTLVTVSS

SEQ ID NO: 55 - protein, 123 aa, synthetic construct
  REGION 1..123: note = 5115-H1-M31
EVQLVESGGGLVQPGGSLRLSCAASGRTFSSFVMSWFRQAPGKEREFVSAISGSGSRARYADSVKGRFTISRDNSKNTLYLQMNSLRAEDTAVYYCAANPRRATPDMRQYAYWGQGTLVTVSS

SEQ ID NO: 56 - protein, 123 aa, synthetic construct
  REGION 1..123: note = 5115-H1-M32
EVQLVESGGGLVQPGGSLRLSCAASGRARSSFVMSWFRQAPGKEREFVSAISGSGSRVRYADSVKGRFTISRDNSKNTLYLQMNSLRAEDTAVYYCAANPRRATPDYTQYAYWGQGTLVTVSS

SEQ ID NO: 57 - protein, 123 aa, synthetic construct
  REGION 1..123: note = 5115-H1-M33
EVQLVESGGGLVQPGGSLRLSCAASMPTFSSFVMSWFRQAPGKEREFVSAISGSGSRSRYADSVKGRFTISRDNSKNTLYLQMNSLRAEDTAVYYCAANPRRATPDYTQYAYWGQGTLVTVSS

SEQ ID NO: 58 - protein, 123 aa, synthetic construct
  REGION 1..123: note = 5115-H1-M34
EVQLVESGGGLVQPGGSLRLSCAASGRTFSSFVMSWFRQAPGKEREFVSAISGSGSRMRYADSVKGRFTISRDNSKNTLYLQMNSLRAEDTAVYYCAANPRRATPDMRQYAYWGQGTLVTVSS

SEQ ID NO: 59 - protein, 123 aa, synthetic construct
  REGION 1..123: note = 5115-H1-M35
EVQLVESGGGLVQPGGSLRLSCAASGRTFSSFVMSWFRQAPGKEREFVSAISGSGSRALYADSVKGRFTISRDNSKNTLYLQMNSLRAEDTAVYYCAANPRRATPDLRQYAYWGQGTLVTVSS

SEQ ID NO: 60 - protein, 123 aa, synthetic construct
  REGION 1..123: note = 5115-H1-M36
EVQLVESGGGLVQPGGSLRLSCAASGRTFPSFVMSWFRQAPGKEREFVSAISGSGSRAYYADSVKGRFTISRDNSKNTLYLQMNSLRAEDTAVYYCAANPRRATPDLRQYAYWGQGTLVTVSS

SEQ ID NO: 61 - protein, 123 aa, synthetic construct
  REGION 1..123: note = 5115-H1-M37
EVQLVESGGGLVQPGGSLRLSCAASGRTFSSFVMAWFRQAPGKGLEFVSAISGKGSRARYADSVKGRFTISRDNSKNTLYLQMNSLRAEDTAVYYCAANPRRATPDLTQYAYWGQGTLVTVSS

SEQ ID NO: 62 - protein, 123 aa, synthetic construct
  REGION 1..123: note = 5115-H1-M38
EVQLVESGGGLVQPGGSLRLSCAASGREFSSFVMAWFRQAPGKGLEFVSAISGKGSRARYADSVKGRFTISRDNSKNTLYLQMNSLRAEDTAVYYCAANPRRATPDLLQYAYWGQGTLVTVSS

SEQ ID NO: 63 - protein, 123 aa, synthetic construct
  REGION 1..123: note = 5115-H1-M39
EVQLVESGGGLVQPGGSLRLSCAASGRTFSSFVMSWFRQAPGKEREFVSAISGSGSRFRYADSVKGRFTISRDNSKNTLYLQMNSLRAEDTAVYYCAANPRRATPDLQQYAYWGQGTLVTVSS

SEQ ID NO: 64 - protein, 123 aa, synthetic construct
  REGION 1..123: note = 5115-H1-M40
EVQLVESGGGLVQPGGSLRLSCAASGRTFSSFVMSWFRQAPGKEREFVSAISGSGSRQRYADSVKGRFTISRDNSKNTLYLQMNSLRAEDTAVYYCAANPRRATPDLRQYAYWGQGTLVTVSS

SEQ ID NO: 65 - protein, 123 aa, synthetic construct
  REGION 1..123: note = 5115-H4-M34-1
EVQLVESGGGLVQPGGSLRLSCAASGRTFNRFVMAWFRQAPGKGLEFVSAISGSGQRARYADSVKGRFTISRDNSKNTLYLQMNSLRAEDTAVYYCAANPRRATPDLTQYAYWGQGTLVTVSS

SEQ ID NO: 66 - protein, 123 aa, synthetic construct
  REGION 1..123: note = 5115-H4-M34-2
EVQLVESGGGLVQPGGSLRLSCAASGRGFSSFVMAWFRQAPGKGLEFVSAISGSGIRARYADSVKGRFTISRDNSKNTLYLQMNSLRAEDTAVYYCAANPRYATPDLTQYAYWGQGTLVTVSS

SEQ ID NO: 67 - protein, 123 aa, synthetic construct
  REGION 1..123: note = 5115-H4-M34-3
EVQLVESGGGLVQPGGSLRLSCAASGGTFSSFVMAWFRQAPGKGLEFVSAISGSGSRARYADSVKGRFTISRDNSKNTLYLQMNSLRAEDTAVYYCAANPRRATPDLTQYKYWGQGTLVTVSS

SEQ ID NO: 68 - protein, 123 aa, synthetic construct
  REGION 1..123: note = 5115-H4-M34-4
EVQLVESGGGLVQPGGSLRLSCAASGGTFSSFVMAWFRQAPGKGLEFVSAISGFGSRARYADSVKGRFTISRDNSKNTLYLQMNSLRAEDTAVYYCAANPRRATPDLTQYAYWGQGTLVTVSS

SEQ ID NO: 69 - protein, 123 aa, synthetic construct
  REGION 1..123: note = 5115-H4-M34-5
EVQLVESGGGLVQPGGSLRLSCAASMTTFSSFVMAWFRQAPGKGLEFVSAISGHGSRARYADSVKGRFTISRDNSKNTLYLQMNSLRAEDTAVYYCAANPRRATPDLTQYAYWGQGTLVTVSS

SEQ ID NO: 70 - protein, 123 aa, synthetic construct
  REGION 1..123: note = 5115-H4-M34-6
EVQLVESGGGLVQPGGSLRLSCAASGRTFSSFVMAWFRQAPGKGLEFVSAISGSGSRSRYADSVKGRFTISRDNSKNTLYLQMNSLRAEDTAVYYCAANPRYATPDLTQYAYWGQGTLVTVSS

SEQ ID NO: 71 - protein, 123 aa, synthetic construct
  REGION 1..123: note = 5115-H4-M34-7
EVQLVESGGGLVQPGGSLRLSCAASGRTFSSFVMAWFRQAPGKGLEFVSAISGSGRQARYADSVKGRFTISRDNSKNTLYLQMNSLRAEDTAVYYCAANPRRATPDLSRYAYWGQGTLVTVSS

SEQ ID NO: 72 - protein, 123 aa, synthetic construct
  REGION 1..123: note = 5115-H4-M34-8
EVQLVESGGGLVQPGGSLRLSCAASGRTFSTFVMAWFRQAPGKGLEFVSAISGSGSRSRYADSVKGRFTISRDNSKNTLYLQMNSLRAEDTAVYYCAANPRRATPDLTQYAYWGQGTLVTVSS

SEQ ID NO: 73 - protein, 123 aa, synthetic construct
  REGION 1..123: note = 5115-H4-M34-9
EVQLVESGGGLVQPGGSLRLSCAASGPAFSSFVMAWFRQAPGKGLEFVSAISGSGSRARYADSVKGRFTISRDNSKNTLYLQMNSLRAEDTAVYYCAANPRRATPDLTQYAYWGQGTLVTVSS

SEQ ID NO: 74 - protein, 123 aa, synthetic construct
  REGION 1..123: note = 5115-H4-M34-10
EVQLVESGGGLVQPGGSLRLSCAASSRTFSSFVMAWFRQAPGKGLEFVSAISGSGTRARYADSVKGRFTISRDNSKNTLYLQMNSLRAEDTAVYYCAANPRRATPDLTAYAYWGQGTLVTVSS

SEQ ID NO: 75 - protein, 123 aa, synthetic construct
  REGION 1..123: note = 5115-H4-M34-11
EVQLVESGGGLVQPGGSLRLSCAASTRTFSSFVMAWFRQAPGKGLEFVSAISGSGSRARYADSVKGRFTISRDNSKNTLYLQMNSLRAEDTAVYYCAANPRRATPDLTQYAYWGQGTLVTVSS

SEQ ID NO: 76 - protein, 123 aa, synthetic construct
  REGION 1..123: note = 5115-H4-M34-12
EVQLVESGGGLVQPGGSLRLSCAASGRPFSSFVMAWFRQAPGKGLEFVSAISGSGSRARYADSVKGRFTISRDNSKNTLYLQMNSLRAEDTAVYYCAANPRYATPDLTQYAYWGQGTLVTVSS

SEQ ID NO: 77 - protein, 123 aa, synthetic construct
  REGION 1..123: note = 5115-H4-M34-13
EVQLVESGGGLVQPGGSLRLSCAASGRTFSSLVMAWFRQAPGKGLEFVSAISGSGMRARYADSVKGRFTISRDNSKNTLYLQMNSLRAEDTAVYYCAANPRRATPDLTQYLYWGQGTLVTVSS

SEQ ID NO: 78 - protein, 123 aa, synthetic construct
  REGION 1..123: note = 5115-H4-M34-14
EVQLVESGGGLVQPGGSLRLSCAASRGTFSSFVMAWFRQAPGKGLEFVSAISGSGKVARYADSVKGRFTISRDNSKNTLYLQMNSLRAEDTAVYYCAANPRRATPDLTQYAYWGQGTLVTVSS

SEQ ID NO: 79 - protein, 123 aa, synthetic construct
  REGION 1..123: note = 5115-H4-M34-15
EVQLVESGGGLVQPGGSLRLSCAASGRTFSSLVMAWFRQAPGKGLEFVSAISGSGSRARYADSVKGRFTISRDNSKNTLYLQMNSLRAEDTAVYYCAANPRRATPDLTQYAYWGQGTLVTVSS

SEQ ID NO: 80 - protein, 123 aa, synthetic construct
  REGION 1..123: note = 5115-H4-M34-16
EVQLVESGGGLVQPGGSLRLSCAASGRTFSSFVMGWFRQAPGKGLEFVSAISGFGSRARYADSVKGRFTISRDNSKNTLYLQMNSLRAEDTAVYYCAANPRRATPDLTQYAYWGQGTLVTVSS

SEQ ID NO: 81 - protein, 6 aa, synthetic construct
  REGION 1..6: note = HCDR1 5115 Contact
SSFVMG

SEQ ID NO: 82 - protein, 10 aa, synthetic construct
  REGION 1..10: note = HCDR1 5115 Abm
GRTFSSFVMG

SEQ ID NO: 83 - protein, 7 aa, synthetic construct
  REGION 1..7: note = HCDR1 5115 Chothia
GRTFSSF

SEQ ID NO: 84 - protein, 8 aa, synthetic construct
  REGION 1..8: note = HCDR1 5115 IMGT
GRTFSSFV

SEQ ID NO: 85 - protein, 5 aa, synthetic construct
  REGION 1..5: note = HCDR1 5115 Kabat+H4-M41+H4-M34-16
SFVMG

SEQ ID NO: 86 - protein, 5 aa, synthetic construct
  REGION 1..5: note = HCDR1 5666
SYVMG

SEQ ID NO: 87 - protein, 5 aa, synthetic construct
  REGION 1..5: note = HCDR1 5115-H0~4+H4-M10+12+25+28+39+44+52+59+69+H1-M1~4+7~23+25~26+28~36+39~40
SFVMS

SEQ ID NO: 88 - protein, 5 aa, synthetic construct
  REGION 1..5: note = HCDR1 5115-H5~6
SFVMM

SEQ ID NO: 89 - protein, 5 aa, synthetic construct
  REGION 1..5: note = HCDR1 5115-H4-M3+34+H1-M5~6+27+37~38+H4-M34-2~7+9~12+14
SFVMA

SEQ ID NO: 90 - protein, 5 aa, synthetic construct
  REGION 1..5: note = HCDR1 5115-H4-M24+28
RFVMS

SEQ ID NO: 91 - protein, 5 aa, synthetic construct
  REGION 1..5: note = HCDR1 5115-H4-M61
SFVLS

SEQ ID NO: 92 - protein, 5 aa, synthetic construct
  REGION 1..5: note = HCDR1 5115-H1-M24
GFVMA

SEQ ID NO: 93 - protein, 5 aa, synthetic construct
  REGION 1..5: note = HCDR1 5115-H4-M34-1
RFVMA

SEQ ID NO: 94 - protein, 5 aa, synthetic construct
  REGION 1..5: note = HCDR1 5115-H4-M34-8
TFVMA

SEQ ID NO: 95 - protein, 5 aa, synthetic construct
  REGION 1..5: note = HCDR1 5115-H4-M34-13+15
SLVMA

SEQ ID NO: 96 - protein, 13 aa, synthetic construct
  REGION 1..13: note = HCDR2 5115 Contact
FVAAISGSGSRAN

SEQ ID NO: 97 - protein, 10 aa, synthetic construct
  REGION 1..10: note = HCDR2 5115 Abm
AISGSGSRAN

SEQ ID NO: 98 - protein, 6 aa, synthetic construct
  REGION 1..6: note = HCDR2 5115 Chothia
SGSGSR

SEQ ID NO: 99 - protein, 8 aa, synthetic construct
  REGION 1..8: note = HCDR2 5115 IMGT
ISGSGSRA

SEQ ID NO: 100 - protein, 17 aa, synthetic construct
  REGION 1..17: note = HCDR2 5115 Kabat +H4-M52
AISGSGSRANYADSVKG

SEQ ID NO: 101 - protein, 17 aa, synthetic construct
  REGION 1..17: note = HCDR2 5666
AISGSGSRSNYADSVKG

SEQ ID NO: 102 - protein, 17 aa, synthetic construct
  REGION 1..17: note = HCDR2 5115-H0~6+H4-M48+H1-M10+29+36
AISGSGSRAYYADSVKG

SEQ ID NO: 103 - protein, 17 aa, synthetic construct
  REGION 1..17: note = HCDR2 5115-H4-M3+24+34+41+44+61+69+H1-M2~3+6+12~13+16+18+23+25+31+H4-M34-3+9+11~12+15
AISGSGSRARYADSVKG

SEQ ID NO: 104 - protein, 17 aa, synthetic construct
  REGION 1..17: note = HCDR2 5115-H4-M10
AISGQGSRSYYADSVKG

SEQ ID NO: 105 - protein, 17 aa, synthetic construct
  REGION 1..17: note = HCDR2 5115-H4-M12
AISGSGSRFYYADSVKG

SEQ ID NO: 106 - protein, 17 aa, synthetic construct
  REGION 1..17: note = HCDR2 5115-H4-M25+35
AISGSGSRALYADSVKG

SEQ ID NO: 107 - protein, 17 aa, synthetic construct
  REGION 1..17: note = HCDR2 5115-H4-M28
AISGGGSRAYYADSVKG

SEQ ID NO: 108 - protein, 17 aa, synthetic construct
  REGION 1..17: note = HCDR2 5115-H4-M39+H1-M1+17+22+33+H4-M34-6+8
AISGSGSRSRYADSVKG

SEQ ID NO: 109 - protein, 17 aa, synthetic construct
  REGION 1..17: note = HCDR2 5115-H4-M59+H1-M7
AISGRGSRAYYADSVKG

SEQ ID NO: 110 - protein, 17 aa, synthetic construct
  REGION 1..17: note = HCDR2 5115-H1-M4+39
AISGSGSRFRYADSVKG

SEQ ID NO: 111 - protein, 17 aa, synthetic construct
  REGION 1..17: note = HCDR2 5115-H1-M5+27
AISGSGLRARYADSVKG

SEQ ID NO: 112 - protein, 17 aa, synthetic construct
  REGION 1..17: note = HCDR2 5115-H1-M8+40
AISGSGSRQRYADSVKG

SEQ ID NO: 113 - protein, 17 aa, synthetic construct
  REGION 1..17: note = HCDR2 5115-H1-M9
AISGSGSRLRYADSVKG

SEQ ID NO: 114 - protein, 17 aa, synthetic construct
  REGION 1..17: note = HCDR2 5115-H1-M11+30
AISGSGSRHRYADSVKG

SEQ ID NO: 115 - protein, 17 aa, synthetic construct
  REGION 1..17: note = HCDR2 5115-H1-M14~15+19+34
AISGSGSRMRYADSVKG

SEQ ID NO: 116 - protein, 17 aa, synthetic construct
  REGION 1..17: note = HCDR2 5115-H1-M20+28
AISGSGSRYRYADSVKG

SEQ ID NO: 117 - protein, 17 aa, synthetic construct
  REGION 1..17: note = HCDR2 5115-H1-M21
AISGSGSRTRYADSVKG

SEQ ID NO: 118 - protein, 17 aa, synthetic construct
  REGION 1..17: note = HCDR2 5115-H1-M24
AISGTGSRARYADSVKG

SEQ ID NO: 119 - protein, 17 aa, synthetic construct
  REGION 1..17: note = HCDR2 5115-H1-M26
AISGSGSRYTYADSVKG

SEQ ID NO: 120 - protein, 17 aa, synthetic construct
  REGION 1..17: note = HCDR2 5115-H1-M32
AISGSGSRVRYADSVKG

SEQ ID NO: 121 - protein, 17 aa, synthetic construct
  REGION 1..17: note = HCDR2 5115-H1-M37~38
AISGKGSRARYADSVKG

SEQ ID NO: 122 - protein, 17 aa, synthetic construct
  REGION 1..17: note = HCDR2 5115-H4-M34-1
AISGSGQRARYADSVKG

SEQ ID NO: 123 - protein, 17 aa, synthetic construct
  REGION 1..17: note = HCDR2 5115-H4-M34-2
AISGSGIRARYADSVKG

SEQ ID NO: 124 - protein, 17 aa, synthetic construct
  REGION 1..17: note = HCDR2 5115-H4-M34-4+16
AISGFGSRARYADSVKG

SEQ ID NO: 125 - protein, 17 aa, synthetic construct
  REGION 1..17: note = HCDR2 5115-H4-M34-5
AISGHGSRARYADSVKG

SEQ ID NO: 126 - protein, 17 aa, synthetic construct
  REGION 1..17: note = HCDR2 5115-H4-M34-7
AISGSGRQARYADSVKG

SEQ ID NO: 127 - protein, 17 aa, synthetic construct
  REGION 1..17: note = HCDR2 5115-H4-M34-10
AISGSGTRARYADSVKG

SEQ ID NO: 128 - protein, 17 aa, synthetic construct
  REGION 1..17: note = HCDR2 5115-H4-M34-13
AISGSGMRARYADSVKG

SEQ ID NO: 129 - protein, 17 aa, synthetic construct
  REGION 1..17: note = HCDR2 5115-H4-M34-14
AISGSGKVARYADSVKG

SEQ ID NO: 130 - protein, 15 aa, synthetic construct
  REGION 1..15: note = HCDR3 5115 Contact
AANPRRATPDYTQYA

SEQ ID NO: 131 - protein, 14 aa, synthetic construct
  REGION 1..14: note = HCDR3 5115 Abm+Chothia+Kabat+H0~H6+H4-M3+H1-M1+4+11+13+20~21+30+32~33
NPRRATPDYTQYAY

SEQ ID NO: 132 - protein, 16 aa, synthetic construct
  REGION 1..16: note = HCDR3 5115 IMGT
AANPRRATPDYTQYAY

SEQ ID NO: 133 - protein, 14 aa, synthetic construct
  REGION 1..14: note = HCDR3 5666
NPRRATTDYTQYAY

SEQ ID NO: 134 - protein, 14 aa, synthetic construct
  REGION 1..14: note = HCDR3 5115-H4-M10+12+24+25+34+44+52+61+69+H1-M3+14+16+18+24+37+H4-M34-1+4+5+8+9+11+14~16
NPRRATPDLTQYAY

SEQ ID NO: 135 - protein, 14 aa, synthetic construct
  REGION 1..14: note = HCDR3 5115-H4-M28+39+48+H1-M7+12+15+29+35+36+40
NPRRATPDLRQYAY

SEQ ID NO: 136 - protein, 14 aa, synthetic construct
  REGION 1..14: note = HCDR3 5115-H4-M41
NPRRATPDYTQYLY

SEQ ID NO: 137 - protein, 14 aa, synthetic construct
  REGION 1..14: note = HCDR3 5115-H4-M59+H1-M23
NPRRATPDMTQYAY

SEQ ID NO: 138 - protein, 14 aa, synthetic construct
  REGION 1..14: note = HCDR3 5115-H1-M2+9+22+38
NPRRATPDLLQYAY

SEQ ID NO: 139 - protein, 14 aa, synthetic construct
  REGION 1..14: note = HCDR3 5115-H1-M5~6
NPRRATPDLTSYAY

SEQ ID NO: 140 - protein, 14 aa, synthetic construct
  REGION 1..14: note = HCDR3 5115-H1-M8
NPRRATPDLSQYAY

SEQ ID NO: 141 - protein, 14 aa, synthetic construct
  REGION 1..14: note = HCDR3 5115-H1-M10
NPRRATPGFTQYAY

SEQ ID NO: 142 - protein, 14 aa, synthetic construct
  REGION 1..14: note = HCDR3 5115-H1-M17
NPRRATPDLIQYAY

SEQ ID NO: 143 - protein, 14 aa, synthetic construct
  REGION 1..14: note = HCDR3 5115-H1-M19
NPRRATPDLHQYAY

SEQ ID NO: 144 - protein, 14 aa, synthetic construct
  REGION 1..14: note = HCDR3 5115-H1-M25
NPRRATPDYSQYAY

SEQ ID NO: 145 - protein, 14 aa, synthetic construct
  REGION 1..14: note = HCDR3 5115-H1-M26
NPRRATPDLMQYAY

SEQ ID NO: 146 - protein, 14 aa, synthetic construct
  REGION 1..14: note = HCDR3 5115-H1-M27+H4-M34-2+6+12
NPRYATPDLTQYAY

SEQ ID NO: 147 - protein, 14 aa, synthetic construct
  REGION 1..14: note = HCDR3 5115-H1-M28
NPRRATPDLKQYAY

SEQ ID NO: 148 - protein, 14 aa, synthetic construct
  REGION 1..14: note = HCDR3 5115-H1-M31+34
NPRRATPDMRQYAY

SEQ ID NO: 149 - protein, 14 aa, synthetic construct
  REGION 1..14: note = HCDR3 5115-H1-M39
NPRRATPDLQQYAY

SEQ ID NO: 150 - protein, 14 aa, synthetic construct
  REGION 1..14: note = HCDR3 5115-H4-M34-3
NPRRATPDLTQYKY

SEQ ID NO: 151 - protein, 14 aa, synthetic construct
  REGION 1..14: note = HCDR3 5115-H4-M34-7
NPRRATPDLSRYAY

SEQ ID NO: 152 - protein, 14 aa, synthetic construct
  REGION 1..14: note = HCDR3 5115-H4-M34-10
NPRRATPDLTAYAY

SEQ ID NO: 153 - protein, 14 aa, synthetic construct
  REGION 1..14: note = HCDR3 5115-H4-M34-13
NPRRATPDLTQYLY

SEQ ID NO: 154 - protein, 29 aa, synthetic construct
  REGION 1..29: note = FR1 5115 Contact
EVQLVESGGGLVQAGGSLRLSCAVSGRTF

SEQ ID NO: 155 - protein, 25 aa, synthetic construct
  REGION 1..25: note = FR1 5115 Abm+Chothia+IMGT
EVQLVESGGGLVQAGGSLRLSCAVS

SEQ ID NO: 156 - protein, 30 aa, synthetic construct
  REGION 1..30: note = FR1 5115+5666 Kabat
EVQLVESGGGLVQAGGSLRLSCAVSGRTFS

SEQ ID NO: 157 - protein, 30 aa, synthetic construct
  REGION 1..30: note = FR1 5115-H0~H6+H4-M3+M12+M28+M34+M39+M41+M61+H1-M1~3+M7~9+M12+M14+M15+M17+M19+M22+M24+M26+M28+M29+M31+M34+M35+M37+M39+M40+H4-M34-6~8+13+15+16
EVQLVESGGGLVQPGGSLRLSCAASGRTFS

SEQ ID NO: 158 - protein, 30 aa, synthetic construct
  REGION 1..30: note = FR1 5115-H4-M10
EVQLVESGGGLVQPGGSLRLSCAASGRSFS

SEQ ID NO: 159 - protein, 30 aa, synthetic construct
  REGION 1..30: note = FR1 5115-H4-M24
EVQLVESSGGLVQPGGSLRLSCAASGRTFS

SEQ ID NO: 160 - protein, 30 aa, synthetic construct
  REGION 1..30: note = FR1 5115-H4-M25
EVQLVESGGGLVQPGGSLRLSCAASGVTFS

SEQ ID NO: 161 - protein, 30 aa, synthetic construct
  REGION 1..30: note = FR1 5115-H4-M44+H1-M18
EVQLVESGGGLVQPGGSLRLSCAASGRRFS

SEQ ID NO: 162 - protein, 30 aa, synthetic construct
  REGION 1..30: note = FR1 5115-H4-M48
EVQLVESGGGLVQPGDSLRLSCAASGRTFS

SEQ ID NO: 163 - protein, 30 aa, synthetic construct
  REGION 1..30: note = FR1 5115-H4-M52+H4-M34-10
EVQLVESGGGLVQPGGSLRLSCAASSRTFS

SEQ ID NO: 164 - protein, 30 aa, synthetic construct
  REGION 1..30: note = FR1 5115-H4-M59
EVQLVESGGGLVQPGGSLRLSCAASGRAFS

SEQ ID NO: 165 - protein, 30 aa, synthetic construct
  REGION 1..30: note = FR1 5115-H4-M69+H1-M20
EVQLVESGGGLVQPGGSLRLSCAASGRTFR

SEQ ID NO: 166 - protein, 30 aa, synthetic construct
  REGION 1..30: note = FR1 5115-H1-M4+M25
EVQLVESGGGLVQPGGSLRLSCAASGRFFS

SEQ ID NO: 167 - protein, 30 aa, synthetic construct
  REGION 1..30: note = FR1 5115-H1-M5
EVQLVESGGGLVQPGGSLRLSCAASGRYFS

SEQ ID NO: 168 - protein, 30 aa, synthetic construct
  REGION 1..30: note = FR1 5115-H1-M6+M38
EVQLVESGGGLVQPGGSLRLSCAASGREFS

SEQ ID NO: 169 - protein, 30 aa, synthetic construct
  REGION 1..30: note = FR1 5115-H1-M10+H4-M34-3+4
EVQLVESGGGLVQPGGSLRLSCAASGGTFS

SEQ ID NO: 170 - protein, 30 aa, synthetic construct
  REGION 1..30: note = FR1 5115-H1-M11
EVQLVESGGGLVQPGGSLRLSCAASGIRFS

SEQ ID NO: 171 - protein, 30 aa, synthetic construct
  REGION 1..30: note = FR1 5115-H1-M13
EVQLVESGGGLVQPGGSLRLSCAASLGTFS

SEQ ID NO: 172 - protein, 30 aa, synthetic construct
  REGION 1..30: note = FR1 5115-H1-M16
EVQLVESGGGLVQPGGSLRLSCAASHRTFS

SEQ ID NO: 173 - protein, 30 aa, synthetic construct
  REGION 1..30: note = FR1 5115-H1-M21
EVQLVESGGGLVQPGGSLRLSCAASGKTFS

SEQ ID NO: 174 - protein, 30 aa, synthetic construct
  REGION 1..30: note = FR1 5115-H1-M23
EVQLVESGGGLVQPGGSLRLSCAASGRTFK

SEQ ID NO: 175 - protein, 30 aa, synthetic construct
  REGION 1..30: note = FR1 5115-H1-M27
EVQLVESGGGLVQPGGSLRLSCAASGRTLS

SEQ ID NO: 176 - protein, 30 aa, synthetic construct
  REGION 1..30: note = FR1 5115-H1-M30
EVQLVESGGGLVQPGGSLRLSCAASGARFS

SEQ ID NO: 177 - protein, 30 aa, synthetic construct
  REGION 1..30: note = FR1 5115-H1-M32
EVQLVESGGGLVQPGGSLRLSCAASGRARS

SEQ ID NO: 178 - protein, 30 aa, synthetic construct
  REGION 1..30: note = FR1 5115-H1-M33
EVQLVESGGGLVQPGGSLRLSCAASMPTFS

SEQ ID NO: 179 - protein, 30 aa, synthetic construct
  REGION 1..30: note = FR1 5115-H1-M36
EVQLVESGGGLVQPGGSLRLSCAASGRTFP

SEQ ID NO: 180 - protein, 30 aa, synthetic construct
  REGION 1..30: note = FR1 5115-H4-M34-1
EVQLVESGGGLVQPGGSLRLSCAASGRTFN

SEQ ID NO: 181 - protein, 30 aa, synthetic construct
  REGION 1..30: note = FR1 5115-H4-M34-2
EVQLVESGGGLVQPGGSLRLSCAASGRGFS

SEQ ID NO: 182 - protein, 30 aa, synthetic construct
  REGION 1..30: note = FR1 5115-H4-M34-5
EVQLVESGGGLVQPGGSLRLSCAASMTTFS

SEQ ID NO: 183 - protein, 30 aa, synthetic construct
  REGION 1..30: note = FR1 5115-H4-M34-9
EVQLVESGGGLVQPGGSLRLSCAASGPAFS

SEQ ID NO: 184 - protein, 30 aa, synthetic construct
  REGION 1..30: note = FR1 5115-H4-M34-11
EVQLVESGGGLVQPGGSLRLSCAASTRTFS

SEQ ID NO: 185 - protein, 30 aa, synthetic construct
  REGION 1..30: note = FR1 5115-H4-M34-12
EVQLVESGGGLVQPGGSLRLSCAASGRPFS

SEQ ID NO: 186 - protein, 30 aa, synthetic construct
  REGION 1..30: note = FR1 5115-H4-M34-14
EVQLVESGGGLVQPGGSLRLSCAASRGTFS

SEQ ID NO: 187 - protein, 11 aa, synthetic construct
  REGION 1..11: note = FR2 5115 Contact
WFRQAPGKERE

SEQ ID NO: 188 - protein, 14 aa, synthetic construct
  REGION 1..14: note = FR2 5115 Abm+Kabat
WFRQAPGKEREFVA

SEQ ID NO: 189 - protein, 19 aa, synthetic construct
  REGION 1..19: note = FR2 5115 Chothia
VMGWFRQAPGKEREFVAAI

SEQ ID NO: 190 - protein, 17 aa, synthetic construct
  REGION 1..17: note = FR2 5115 IMGT
MGWFRQAPGKEREFVAA

SEQ ID NO: 191 - protein, 14 aa, synthetic construct
  REGION 1..14: note = FR2 5666
WFRQAPGKERELVA

SEQ ID NO: 192 - protein, 14 aa, synthetic construct
  REGION 1..14: note = FR2 5115-H0+H1+H6+H1-M1~M4+M7~M23+M25+M26+M28~M36+M39+M40
WFRQAPGKEREFVS

SEQ ID NO: 193 - protein, 14 aa, synthetic construct
  REGION 1..14: note = FR2 5115-H2
WFRQAPGKGREFVS

SEQ ID NO: 194 - protein, 14 aa, synthetic construct
  REGION 1..14: note = FR2 5115-H3
WFRQAPGKELEFVS

SEQ ID NO: 195 - protein, 14 aa, synthetic construct
  REGION 1..14: note = FR2 5115-H4+H5+H4-M+H1-M5+M6+M24+M27+M37+M38+H4-M34-1~16
WFRQAPGKGLEFVS

SEQ ID NO: 196 - protein, 37 aa, synthetic construct
  REGION 1..37: note = FR3 5115 Contact
YADSVKGRFTVSRDNANNTVYLQMNSLKPDDTALYYC

SEQ ID NO: 197 - protein, 39 aa, synthetic construct
  REGION 1..39: note = FR3 5115 Abm
YADSVKGRFTVSRDNANNTVYLQMNSLKPDDTALYYCAA

SEQ ID NO: 198 - protein, 41 aa, synthetic construct
  REGION 1..41: note = FR3 5115 Chothia
ANYADSVKGRFTVSRDNANNTVYLQMNSLKPDDTALYYCAA

SEQ ID NO: 199 - protein, 38 aa, synthetic construct
  REGION 1..38: note = FR3 5115 IMGT
NYADSVKGRFTVSRDNANNTVYLQMNSLKPDDTALYYC

SEQ ID NO: 200 - protein, 32 aa, synthetic construct
  REGION 1..32: note = FR3 5115 Kabat
RFTVSRDNANNTVYLQMNSLKPDDTALYYCAA

SEQ ID NO: 201 - protein, 32 aa, synthetic construct
  REGION 1..32: note = FR3 5666
RFTVSRDNANNTVYLQMSSLRPDDTGLYYCAA

SEQ ID NO: 202 - protein, 32 aa, synthetic construct
  REGION 1..32: note = FR3 5115+H0~H6+H4-M3+10+12+24+25+34+39+41+44+48+52+59+61+69+H1-M1~M40+H4-M34-1~16
RFTISRDNSKNTLYLQMNSLRAEDTAVYYCAA

SEQ ID NO: 203 - protein, 32 aa, synthetic construct
  REGION 1..32: note = FR3 5115-H4-M28
RFAISRDNSKNTLYLQMNSLRAEDTAVYYCAA

SEQ ID NO: 204 - protein, 12 aa, synthetic construct
  REGION 1..12: note = FR4 5115 Contact
YWGQGTQVTVSS

SEQ ID NO: 205 - protein, 11 aa, synthetic construct
  REGION 1..11: note = FR4 5115+5666
WGQGTQVTVSS

SEQ ID NO: 206 - protein, 11 aa, synthetic construct
  REGION 1..11: note = FR4 5115-H
WGQGTLVTVSS

SEQ ID NO: 207 - protein, 449 aa, synthetic construct
  REGION 1..449: note = Teprotumumab HC
QVQLVQSGAEVKKPGASVKVSCKASGYSFTSSWIHWVKQAPGQGLEWMGEINPGNVRTNYNENFRNKVTMTVDTSISTAYMELSRLRSDDTAVYYCTVVFYGEPYFPYWGQGTLVTVSSASTKGPSVFPLAPSSKSTSGGTAALGCLVKDYFPEPVTVSWNSGALTSGVHTFPAVLQSSGLYSLSSVVTVPSSSLGTQTYICNVNHKPSNTKVDKRVEPKSCDKTHTCPPCPAPEAAGGPSVFLFPPKPKDTLMISRTPEVTCVVVDVSHEDPEVKFNWYVDGVEVHNAKTKPREEQYNSTYRVVSVLTVLHQDWLNGKEYKCKVSNKALPAPIEKTISKAKGQPREPQVYTLPPSREEMTKNQVSLTCLVKGFYPSDIAVEWESNGQPENNYKTTPPVLDSDGSFFLYSKLTVDKSRWQQGNVFSCSVMHEALHNHYTQKSLSLSPGK

SEQ ID NO: 208 - protein, 215 aa, synthetic construct
  REGION 1..215: note = Teprotumumab LC
QIVLTQSPGTLSLSPGERATMTCTASSSVSSSYFHWYQQKPGQAPRLWIYRTSRLASGVPDRFSGSGSGTDFTLTISRLEPEDAATYYCHQFHRSPLTFGAGTKLEIKRTVAAPSVFIFPPSDEQLKSGTASVVCLLNNFYPREAKVQWKVDNALQSGNSQESVTEQDSKDSTYSLSSTLTLSKADYEKHKVYACEVTHQGLSSPVTKSFNRGEC

SEQ ID NO: 209 - protein, 232 aa, synthetic construct
  REGION 1..232: note = Fc IgG1
EPKSCDKTHTCPPCPAPELLGGPSVFLFPPKPKDTLMISRTPEVTCVVVDVSHEDPEVKFNWYVDGVEVHNAKTKPREEQYNSTYRVVSVLTVLHQDWLNGKEYKCKVSNKALPAPIEKTISKAKGQPREPQVYTLPPSRDELTKNQVSLTCLVKGFYPSDIAVEWESNGQPENNYKTTPPVLDSDGSFFLYSKLTVDKSRWQQGNVFSCSVMHEALHNHYTQKSLSLSPGK

SEQ ID NO: 210 - protein, 232 aa, synthetic construct
  REGION 1..232: note = Fc IgG1 D356E L358M
EPKSCDKTHTCPPCPAPELLGGPSVFLFPPKPKDTLMISRTPEVTCVVVDVSHEDPEVKFNWYVDGVEVHNAKTKPREEQYNSTYRVVSVLTVLHQDWLNGKEYKCKVSNKALPAPIEKTISKAKGQPREPQVYTLPPSREEMTKNQVSLTCLVKGFYPSDIAVEWESNGQPENNYKTTPPVLDSDGSFFLYSKLTVDKSRWQQGNVFSCSVMHEALHNHYTQKSLSLSPGK

SEQ ID NO: 211 - protein, 232 aa, synthetic construct
  REGION 1..232: note = Fc' IgG1 C220S L234A L235A D356E L358M
EPKSSDKTHTCPPCPAPEAAGGPSVFLFPPKPKDTLMISRTPEVTCVVVDVSHEDPEVKFNWYVDGVEVHNAKTKPREEQYNSTYRVVSVLTVLHQDWLNGKEYKCKVSNKALPAPIEKTISKAKGQPREPQVYTLPPSREEMTKNQVSLTCLVKGFYPSDIAVEWESNGQPENNYKTTPPVLDSDGSFFLYSKLTVDKSRWQQGNVFSCSVMHEALHNHYTQKSLSLSPGK

SEQ ID NO: 212 - protein, 232 aa, synthetic construct
  REGION 1..232: note = Fc" IgG1 C220A L234A L235A D356E L358M
EPKSADKTHTCPPCPAPEAAGGPSVFLFPPKPKDTLMISRTPEVTCVVVDVSHEDPEVKFNWYVDGVEVHNAKTKPREEQYNSTYRVVSVLTVLHQDWLNGKEYKCKVSNKALPAPIEKTISKAKGQPREPQVYTLPPSREEMTKNQVSLTCLVKGFYPSDIAVEWESNGQPENNYKTTPPVLDSDGSFFLYSKLTVDKSRWQQGNVFSCSVMHEALHNHYTQKSLSLSPGK

SEQ ID NO: 213-214 - skipped (2 entries)

SEQ ID NO: 215 - protein, 17 aa, synthetic construct
  REGION 1..17: note = HCDR2 A
  SITE 5: note = misc_feature - Xaa = Phe, Gly, His, Lys, Gln, Arg, Ser or Thr
  SITE 7: note = misc_feature - Xaa = Ile, Lys, Leu, Met, Gln, Arg, Ser or Thr
  SITE 8: note = misc_feature - Xaa = Gln, Arg or Val
  SITE 9: note = misc_feature - Xaa = Ala, Phe, His, Leu, Met, Gln, Ser, Thr, Val or Tyr
  SITE 10: note = misc_feature - Xaa = Leu, Asn, Arg, Thr or Tyr
AISGXGXXXXYADSVKG

SEQ ID NO: 216 - protein, 17 aa, synthetic construct
  REGION 1..17: note = HCDR2 B
  SITE 7: note = misc_feature - Xaa = Met or Ser
  SITE 10: note = misc_feature - Xaa = Arg or Tyr
AISGSGXRAXYADSVKG

SEQ ID NO: 217 - protein, 14 aa, synthetic construct
  REGION 1..14: note = HCDR3 A
  SITE 4: note = misc_feature - Xaa = Arg or Tyr
  SITE 7: note = misc_feature - Xaa = Pro or Thr
  SITE 8: note = misc_feature - Xaa = Asp or Gly
  SITE 9: note = misc_feature - Xaa = Phe, Leu, Met or Tyr
  SITE 10: note = misc_feature - Xaa = His, Ile, Lys, Leu, Met, Gln, Arg, Ser or Thr
  SITE 11: note = misc_feature - Xaa = Ala, Gln, Arg or Ser
  SITE 13: note = misc_feature - Xaa = Ala, Lys or Leu
NPRXATXXXXXYXY

SEQ ID NO: 218 - protein, 14 aa, synthetic construct
  REGION 1..14: note = HCDR3 B
  SITE 9: note = misc_feature - Xaa = Leu or Tyr
  SITE 13: note = misc_feature - Xaa = Ala or Leu
NPRRATPDXTQYXY

SEQ ID NO: 219 - protein, 30 aa, synthetic construct
  REGION 1..30: note = FR1 A
  SITE 8: note = misc_feature - Xaa = Gly or Ser
  SITE 14: note = misc_feature - Xaa = Ala or Pro
  SITE 16: note = misc_feature - Xaa = Asp or Gly
  SITE 24: note = misc_feature - Xaa = Ala or Val
  SITE 26: note = misc_feature - Xaa = Gly, His, Leu, Met, Arg, Ser or Thr
  SITE 27: note = misc_feature - Xaa = Ala, Gly, Ile, Lys, Pro, Arg, Thr or Val
  SITE 28: note = misc_feature - Xaa = Ala, Glu, Phe, Gly, Pro, Arg, Ser, Thr or Tyr
  SITE 29: note = misc_feature - Xaa = Phe, Leu or Arg
  SITE 30: note = misc_feature - Xaa = Lys, Asn, Pro, Arg or Ser
EVQLVESXGGLVQXGXSLRLSCAXSXXXXX

SEQ ID NO: 220 - protein, 30 aa, synthetic construct
  REGION 1..30: note = FR1 B
  SITE 30: note = misc_feature - Xaa = Arg or Ser
EVQLVESGGGLVQPGGSLRLSCAASGRTFX

SEQ ID NO: 221 - protein, 14 aa, synthetic construct
  REGION 1..14: note = FR2 A
  SITE 9: note = misc_feature - Xaa = Glu or Gly
  SITE 10: note = misc_feature - Xaa = Leu or Arg
  SITE 12: note = misc_feature - Xaa = Phe or Leu
  SITE 14: note = misc_feature - Xaa = Ala or Ser
WFRQAPGKXXEXVX

SEQ ID NO: 222 - protein, 14 aa, synthetic construct
  REGION 1..14: note = FR2 B
  SITE 9: note = misc_feature - Xaa = Glu or Gly
  SITE 10: note = misc_feature - Xaa = Leu or Arg
WFRQAPGKXXEFVS

SEQ ID NO: 223 - protein, 32 aa, synthetic construct
  REGION 1..32: note = FR3 A
  SITE 3: note = misc_feature - Xaa = Ala or Thr
  SITE 4: note = misc_feature - Xaa = Ile or Val
  SITE 9: note = misc_feature - Xaa = Ala or Ser
  SITE 10: note = misc_feature - Xaa = Lys or Asn
  SITE 13: note = misc_feature - Xaa = Leu or Val
  SITE 18: note = misc_feature - Xaa = Asn or Ser
  SITE 21: note = misc_feature - Xaa = Lys or Arg
  SITE 22: note = misc_feature - Xaa = Ala or Pro
  SITE 23: note = misc_feature - Xaa = Asp or Glu
  SITE 26: note = misc_feature - Xaa = Ala or Gly
  SITE 27: note = misc_feature - Xaa = Leu or Val
RFXXSRDNXXNTXYLQMXSLXXXDTXXYYCAA

SEQ ID NO: 224 - protein, 11 aa, synthetic construct
  REGION 1..11: note = FR4 A
  SITE 6: note = misc_feature - Xaa = Leu or Gln
WGQGTXVTVSS

SEQ ID NO: 225 - protein, 123 aa, synthetic construct
  REGION 1..123: note = VH A
  SITE 8: note = misc_feature - Xaa = Gly or Ser
  SITE 14: note = misc_feature - Xaa = Ala or Pro
  SITE 16: note = misc_feature - Xaa = Asp or Gly
  SITE 24: note = misc_feature - Xaa = Ala or Val
  SITE 26: note = misc_feature - Xaa = Gly, His, Leu, Met, Arg, Ser or Thr
  SITE 27: note = misc_feature - Xaa = Ala, Gly, Ile, Lys, Pro, Arg, Thr or Val
  SITE 28: note = misc_feature - Xaa = Ala, Glu, Phe, Gly, Pro, Arg, Ser, Thr or Tyr
  SITE 29: note = misc_feature - Xaa = Phe, Leu or Arg
  SITE 30: note = misc_feature - Xaa = Lys, Asn, Pro, Arg or Ser
  SITE 31: note = misc_feature - Xaa = Gly, Arg, Ser or Thr
  SITE 32: note = misc_feature - Xaa = Phe, Leu or Tyr
  SITE 34: note = misc_feature - Xaa = Leu or Met
  SITE 35: note = misc_feature - Xaa = Ala, Gly, Met or Ser
  SITE 44: note = misc_feature - Xaa = Glu or Gly
  SITE 45: note = misc_feature - Xaa = Leu or Arg
  SITE 47: note = misc_feature - Xaa = Phe or Leu
  SITE 49: note = misc_feature - Xaa = Ala or Ser
  SITE 54: note = misc_feature - Xaa = Phe, Gly, His, Lys, Gln, Arg, Ser or Thr
  SITE 56: note = misc_feature - Xaa = Ile, Lys, Leu, Met, Gln, Arg, Ser or Thr
  SITE 57: note = misc_feature - Xaa = Gln, Arg or Val
  SITE 58: note = misc_feature - Xaa = Ala, Phe, His, Leu, Met, Gln, Ser, Thr, Val or Tyr
  SITE 59: note = misc_feature - Xaa = Leu, Asn, Arg, Thr or Tyr
  SITE 69: note = misc_feature - Xaa = Ala or Thr
  SITE 70: note = misc_feature - Xaa = Ile or Val
  SITE 75: note = misc_feature - Xaa = Ala or Ser
  SITE 76: note = misc_feature - Xaa = Lys or Asn
  SITE 79: note = misc_feature - Xaa = Leu or Val
  SITE 84: note = misc_feature - Xaa = Asn or Ser
  SITE 87: note = misc_feature - Xaa = Lys or Arg
  SITE 88: note = misc_feature - Xaa = Ala or Pro
  SITE 89: note = misc_feature - Xaa = Asp or Glu
  SITE 92: note = misc_feature - Xaa = Ala or Gly
  SITE 93: note = misc_feature - Xaa = Leu or Val
  SITE 102: note = misc_feature - Xaa = Arg or Tyr
  SITE 105: note = misc_feature - Xaa = Pro or Thr
  SITE 106: note = misc_feature - Xaa = Asp or Gly
  SITE 107: note = misc_feature - Xaa = Phe, Leu, Met or Tyr
  SITE 108: note = misc_feature - Xaa = His, Ile, Lys, Leu, Met, Gln, Arg, Ser or Thr
  SITE 109: note = misc_feature - Xaa = Ala, Gln, Arg or Ser
  SITE 111: note = misc_feature - Xaa = Ala, Lys or Leu
  SITE 118: note = misc_feature - Xaa = Leu or Gln
EVQLVESXGGLVQXGXSLRLSCAXSXXXXXXXVXXWFRQAPGKXXEXVXAISGXGXXXXYADSVKGRFXXSRDNXXNTXYLQMXSLXXXDTXXYYCAANPRXATXXXXXYXYWGQGTXVTVSS

SEQ ID NO: 226 - protein, 123 aa, synthetic construct; identical to SEQ ID NO: 225
  REGION 1..123: note = VH B
  SITE 8: note = misc_feature - Xaa = Ala, Gly or Ser
  SITE 14: note = misc_feature - Xaa = Ala or Pro
  SITE 16: note = misc_feature - Xaa = Asp or Gly
  SITE 24: note = misc_feature - Xaa = Ala or Val
  SITE 26: note = misc_feature - Xaa = Gly, His, Leu, Met, Arg, Ser or Thr
  SITE 27: note = misc_feature - Xaa = Ala, Gly, Ile, Lys, Pro, Arg, Thr or Val
  SITE 28: note = misc_feature - Xaa = Ala, Glu, Phe, Gly, Pro, Arg, Ser, Thr or Tyr
  SITE 29: note = misc_feature - Xaa = Phe, Leu or Arg
  SITE 30: note = misc_feature - Xaa = Lys, Asn, Pro, Arg or Ser
  SITE 31: note = misc_feature - Xaa = Gly, Arg, Ser or Thr
  SITE 32: note = misc_feature - Xaa = Phe, Leu or Tyr
  SITE 34: note = misc_feature - Xaa = Leu or Met
  SITE 35: note = misc_feature - Xaa = Ala, Gly, Met or Ser
  SITE 44: note = misc_feature - Xaa = Glu or Gly
  SITE 45: note = misc_feature - Xaa = Leu or Arg
  SITE 47: note = misc_feature - Xaa = Phe or Leu
  SITE 49: note = misc_feature - Xaa = Ala or Ser
  SITE 54: note = misc_feature - Xaa = Phe, Gly, His, Lys, Gln, Arg, Ser or Thr
  SITE 56: note = misc_feature - Xaa = Ile, Lys, Leu, Met, Gln, Arg, Ser or Thr
  SITE 57: note = misc_feature - Xaa = Gln, Arg or Val
  SITE 58: note = misc_feature - Xaa = Ala, Phe, His, Leu, Met, Gln, Ser, Thr, Val or Tyr
  SITE 59: note = misc_feature - Xaa = Leu, Asn, Arg, Thr or Tyr
  SITE 69: note = misc_feature - Xaa = Ala or Thr
  SITE 70: note = misc_feature - Xaa = Ile or Val
  SITE 75: note = misc_feature - Xaa = Ala or Ser
  SITE 76: note = misc_feature - Xaa = Lys or Asn
  SITE 79: note = misc_feature - Xaa = Leu or Val
  SITE 84: note = misc_feature - Xaa = Asn or Ser
  SITE 87: note = misc_feature - Xaa = Lys or Arg
  SITE 88: note = misc_feature - Xaa = Ala or Pro
  SITE 89: note = misc_feature - Xaa = Asp or Glu
  SITE 92: note = misc_feature - Xaa = Ala or Gly
  SITE 93: note = misc_feature - Xaa = Leu or Val
  SITE 102: note = misc_feature - Xaa = Arg or Tyr
  SITE 105: note = misc_feature - Xaa = Pro or Thr
  SITE 106: note = misc_feature - Xaa = Asp or Gly
  SITE 107: note = misc_feature - Xaa = Phe, Leu, Met or Tyr
  SITE 108: note = misc_feature - Xaa = His, Ile, Lys, Leu, Met, Gln, Arg, Ser or Thr
  SITE 109: note = misc_feature - Xaa = Ala, Gln, Arg or Ser
  SITE 111: note = misc_feature - Xaa = Ala, Lys or Leu
  SITE 118: note = misc_feature - Xaa = Leu or Gln

SEQ ID NO: 227 - protein, 232 aa, synthetic construct
  REGION 1..232: note = Fc A
  SITE 5: note = misc_feature - Xaa = Ala, Cys or Ser
  SITE 19: note = misc_feature - Xaa = Ala or Leu
  SITE 20: note = misc_feature - Xaa = Ala or Leu
  SITE 141: note = misc_feature - Xaa = Asp or Glu
  SITE 143: note = misc_feature - Xaa = Leu or Met
EPKSXDKTHTCPPCPAPEXXGGPSVFLFPPKPKDTLMISRTPEVTCVVVDVSHEDPEVKFNWYVDGVEVHNAKTKPREEQYNSTYRVVSVLTVLHQDWLNGKEYKCKVSNKALPAPIEKTISKAKGQPREPQVYTLPPSRXEXTKNQVSLTCLVKGFYPSDIAVEWESNGQPENNYKTTPPVLDSDGSFFLYSKLTVDKSRWQQGNVFSCSVMHEALHNHYTQKSLSLSPGK